European Patent Application EP 4 364 583 A1, published May 8, 2024. Title: Composition comprising 3 strains of Lactobacillus sp. and use thereof. Applicant: GIBIOME. The sequence listing filed with the application follows.

SEQUENCE LISTING (5 sequences)

SEQ ID NO: 1 - DNA, 1441 bp, Artificial Sequence
  GB102 rRNA
gcaagtcgaacgcgttggcccaattgattgatggtgcttgcacctgattgattttggtcgccaacgagtggcggacgggtgagtaacacgtaggtaacctgcccagaagcgggggacaacatttggaaacagatgctaataccgcataacaacgttgttcgcatgaacaacgcttaaaagatggcttctcgctatcacttctggatggacctgcggtgcattagcttgttggtggggtaatggcctaccaaggcgatgatgcatagccgagttgagagactgatcggccacaatgggactgagacacggcccatactcctacgggaggcagcagtagggaatcttccacaatgggcgcaagcctgatggagcaacaccgcgtgagtgaagaagggtttcggctcgtaaagctctgttgttaaagaagaacacgtatgagagtaactgttcatacgttgacggtatttaaccagaaagtcacggctaactacgtgccagcagccgcggtaatacgtaggtggcaagcgttatccggatttattgggcgtaaagagagtgcaggcggttttctaagtctgatgtgaaagccttcggcttaaccggagaagtgcatcggaaactggataacttgagtgcagaagagggtagtggaactccatgtgtagcggtggaatgcgtagatatatggaagaacaccagtggcgaaggcggctacctggtctgcaactgacgctgagactcgaaagcatgggtagcgaacaggattagataccctggtagtccatgccgtaaacgatgagtgctaggtgttggagggtttccgcccttcagtgccggagctaacgcattaagcactccgcctggggagtacgaccgcaaggttgaaactcaaaggaattgacgggggcccgcacaagcggtggagcatgtggtttaattcgaagctacgcgaagaaccttaccaggtcttgacatcttgcgccaaccctagagatagggcgtttccttcgggaacgcaatgacaggtggtgcatggtcgtcgtcagctcgtgtcgtgagatgttgggttaagtcccgcaacgagcgcaacccttgttactagttgccagcattaagttgggcactctagtgagactgccggtgacaaaccggaggaaggtggggacgacgtcagatcatcatgccccttatgacctgggctacacacgtgctacaatggacggtacaacgagtcgcgaactcgcgagggcaagcaaatctcttaaaaccgttctcagttcggactgcaggctgcaactcgcctgcacgaagtcggaatcgctagtaatcgcggatcagcatgccgcggtgaatacgttcccgggccttgtacacaccgcccgtcacaccatgagagtttgtaacacccaaagtcggtggggtaaccttttaggagccagcc

SEQ ID NO: 2 - DNA, 1447 bp, Artificial Sequence
  GB103 rRNA
atacatgcaagtcgaacgcgttggcccaattgattgatggtgcttgcacctgattgattttggtcgccaacgagtggcggacgggtgagtaacacgtaggtaacctgcccagaagcgggggacaacatttggaaacagatgctaataccgcataacagcgttgttcgcatgaacaacgcttaaaagatggcttctcgctatcacttctggatggacctgcggtgcattagcttgttggtggggtaacggcctaccaaggcgatgatgcatagccgagttgagagactgatcggccacaatgggactgagacacggcccatactcctacgggaggcagcagtagggaatcttccacaatgggcgcaagcctgatggagcaacaccgcgtgagtgaagaagggtttcggctcgtaaagctctgttgttaaagaagaacacgtatgagagtaactgttcatacgttgacggtatttaaccagaaagtcacggctaactacgtgccagcagccgcggtaatacgtaggtggcaagcgttatccggatttattgggcgtaaagagagtgcaggcggttttctaagtctgatgtgaaagccttcggcttaaccggagaagtgcatcggaaactggataacttgagtgcagaagagggtagtggaactccatgtgtagcggtggaatgcgtagatatatggaagaacaccagtggcgaaggcggctacctggtctgcaactgacgctgagactcgaaagcatgggtagcgaacaggattagataccctggtagtccatgccgtaaacgatgagtgctaggtgttggagggtttccgcccttcagtgccggagctaacgcattaagcactccgcctggggagtacgaccgcaaggttgaaactcaaaggaattgacgggggcccgcacaagcggtggagcatgtggtttaattcgaagctacgcgaagaaccttaccaggtcttgacatcttgcgccaaccctagagatagggcgtttccttcgggaacgcaatgacaggtggtgcatggtcgtcgtcagctcgtgtcgtgagatgttgggttaagtcccgcaacgagcgcaacccttgttactagttgccagcattaagttgggcactctagtgagactgccggtgacaaaccggaggaaggtggggacgacgtcagatcatcatgccccttatgacctgggctacacacgtgctacaatggacggtacaacgagtcgcgaactcgcgagggcaagcaaatctcttaaaaccgttctcagttcggactgcaggctgcaactcgcctgcacgaagtcggaatcgctagtaatcgcggatcagcatgccgcggtgaatacgttcccgggccttgtacacaccgcccgtcacaccatgagagtttgtaacacccaaagtcggtggggtaaccttttaggagccagcc

SEQ ID NO: 3 - DNA, 1552 bp, Artificial Sequence
  GB104 rRNA
agagtttgatcctggctcaggacgaacgctggcggcgtgcctaatacatgcaagtcgaacgaactctggtattgattggtgcttgcatcatgatttacatttgagtgagtggcgaactggtgagtaacacgtgggaaacctgcccagaagcgggggataacacctggaaacagatgctaataccgcataacaacttggaccgcatggtccgagtttgaaagatggctttggctatcacttttggatggtcccgcggcgtattagctagatggtggggtaacggctcaccatggcaatgatacgtagccgacctgagagggtaatcggccacattgggactgagacacggcccaaactcctacgggaggcagcagtagggaatcttccacaatggacgaaagtctgatggagcaacgccgcgtgagtgaagaagggtttcggctcgtaaaactctgttgttaaagaagaacatatctgagagtaactgttcaggtattgacggtatttaaccagaaagccacggctaactacgtgccagcagccgcggtaatacgtaggtggcaagcgttgtccggatttattgggcgtaaagcgagcgcaggcggttttttaagtctgatgtgaaagccttcggctcaaccgaagaagtgcatcggaaactgggaaacttgagtgcagaagaggacagtggaactccatgtgtagcggtgaaatgcgtagatatatggaagaacaccagtggcgaaggcggctgtctggtctgtaactgacgctgaggctcgaaagtatgggtagcaaacaggattagataccctggtagtccataccgtaaacgatgaatgctaagtgttggagggtttccgcccttcagtgctgcagctaacgcattaagcattccgcctgggagtacggccgcaaggctgaaactcaaaggaattgacgggggcccgcacaagcggtggagcatgtggtttaattcgaagctacgcgaagaaccttaccaggtcttgacatactatgcaaatctaagagattagacgttcccttcggggacatggatacaggtggtgcatggttgtcgtcagctcgtgtcgtgagatgttgggttaagtcccgcaacgagcgcaacccttattatcagttgccagcattaagttgggcactctggtgagactgccggtgacaaaccggaggaaggtgggatgacgtcaaatcatcatgccccttatgacctgggctacacacgtgctacaatggatggtacaacgagttgcgaactcgcgagagtaagctaatctcttaaagccattctcagttcggattgtaggctgcaactcgcctacatgaagtcggaatcgctagtaatcgcggatcagcatgccgcggtgaatacgttcccgggccttgtacacaccgcccgtcacaccatgagagtttgtaacacccaaagtcggtgggtaaccttttaggaaccagccgcctaaggtgggacagatgattagggtgaagtcgtaacaaggtagccgtaggagaacctgcggctggatcacct

SEQ ID NO: 4 - DNA, 17 bp, Artificial Sequence
  Primer_341F
cctacgggnggcwgcag

SEQ ID NO: 5 - DNA, 21 bp, Artificial Sequence
  Primer_805R
gactachvgggtatctaatcc